European Patent Application EP 4 159 750 A1, published April 5, 2023. Title: DUAL-AGONIST COMPOUND FOR BOTH GLP-1 AND GIP RECEPTORS AND APPLICATION THEREOF. Applicant: BEIJING TUO JIE BIOPHARMACEUTICAL CO. LTD. Application EP 21812549.0. The sequence listing filed with the application follows.

SEQUENCE LISTING (20 sequences)

SEQ ID NO: 1 - protein, 39 aa, artificial sequence
  VARIANT (2)..(2): Xaa is Aib
YXEGTFTSDYSIYKDKIAAQEFVNWLIAGGPSSGAPPPS

SEQ ID NO: 2 - protein, 39 aa, artificial sequence
  VARIANT (2)..(2): Xaa is Aib
YXEGTFTSDYSIYKDRIAAQEFVNWLIAGGPSSGAPPPS

SEQ ID NO: 3 - protein, 39 aa, artificial sequence
  VARIANT (2)..(2): Xaa is Aib
YXEGTFTSDYSIYKDKIAAQEFINWLIAGGPSSGAPPPS

SEQ ID NO: 4 - protein, 39 aa, artificial sequence
  VARIANT (2)..(2): Xaa is Aib
YXEGTFTSDYSIYKDRIAAQEFINWLIAGGPSSGAPPPS

SEQ ID NO: 5 - protein, 39 aa, artificial sequence
  VARIANT (2)..(2): Xaa is Aib
YXEGTFTSDYSIYKDKIAAQEFINWLLAGGPSSGAPPPS

SEQ ID NO: 6 - protein, 39 aa, artificial sequence
  VARIANT (2)..(2): Xaa is Aib
YXEGTFTSDYSIYKDRIAAQEFVNWLLAGGPSSGAPPPS

SEQ ID NO: 7 - protein, 39 aa, artificial sequence
  VARIANT (2)..(2): Xaa is Aib
YXEGTFTSDYSIYKDKIAAQEFVNWLLAGGPSSGAPPPS

SEQ ID NO: 8 - protein, 39 aa, artificial sequence
  VARIANT (2)..(2): Xaa is Aib
YXEGTFTSDYSIYLEKIAAQEFVNWLLAGGPSSGAPPPS

SEQ ID NO: 9 - protein, 39 aa, artificial sequence
  VARIANT (2)..(2): Xaa is Aib
YXEGTFTSDYSIYLEKIAAQEFVNWLIAGGPSSGAPPPS

SEQ ID NO: 10 - protein, 39 aa, artificial sequence
  VARIANT (2)..(2): Xaa is Aib
YXEGTFTSDYSIYLEKIAAQEFINWLIAGGPSSGAPPPS

SEQ ID NO: 11 - protein, 39 aa, artificial sequence
  VARIANT (2)..(2): Xaa is Aib
YXEGTFTSDYSIYLEKIAAQEFINWLLAGGPSSGAPPPS

SEQ ID NO: 12 - protein, 39 aa, artificial sequence
  VARIANT (2)..(2): Xaa is Aib
YXEGTFTSDYSIYKEKIAAQEFVNWLIAGGPSSGAPPPS

SEQ ID NO: 13 - protein, 39 aa, artificial sequence
  VARIANT (2)..(2): Xaa is Aib
YXEGTFTSDYSIYKERIAAQEFVNWLIAGGPSSGAPPPS

SEQ ID NO: 14 - protein, 39 aa, artificial sequence
  VARIANT (2)..(2): Xaa is Aib
YXEGTFTSDYSIYKEKIAAQEFINWLIAGGPSSGAPPPS

SEQ ID NO: 15 - protein, 39 aa, artificial sequence
  VARIANT (2)..(2): Xaa is Aib
YXEGTFTSDYSIYKERIAAQEFINWLIAGGPSSGAPPPS

SEQ ID NO: 16 - protein, 39 aa, artificial sequence
  VARIANT (2)..(2): Xaa is Aib
YXEGTFTSDYSIYKEKIAAQEFINWLLAGGPSSGAPPPS

SEQ ID NO: 17 - protein, 39 aa, artificial sequence
  VARIANT (2)..(2): Xaa is Aib
YXEGTFTSDYSIYKERIAAQEFVNWLLAGGPSSGAPPPS

SEQ ID NO: 18 - protein, 39 aa, artificial sequence
  VARIANT (2)..(2): Xaa is Aib
YXEGTFTSDYSIYKEKIAAQEFVNWLLAGGPSSGAPPPS

SEQ ID NO: 19 - protein, 39 aa, Artificial Sequence
  VARIANT (1)..(1): Xaa is selected from the group consisting of Tyr and His
  VARIANT (2)..(2): Xaa is selected from the group consisting of Aib and D-Ala
  VARIANT (10)..(10): Xaa is selected from the group consisting of Val and Tyr
  VARIANT (12)..(12): Xaa is selected from the group consisting of Ser and Ile
  VARIANT (13)..(13): Xaa is selected from the group consisting of Tyr and Ala
  VARIANT (14)..(14): Xaa is selected from the group consisting of Leu and Nle
  VARIANT (15)..(15): Xaa is selected from the group consisting of Asp and Glu
  VARIANT (16)..(16): Xaa is selected from the group consisting of Arg, Glu, Gly, Lys and Aib
  VARIANT (17)..(17): Xaa is selected from the group consisting of Glu, Ile and Gln
  VARIANT (18)..(18): Xaa is selected from the group consisting of Ala, Aib and His
  VARIANT (19)..(19): Xaa is selected from the group consisting of Ala, Aib and Gln
  VARIANT (20)..(20): Xaa is selected from the group consisting of Gln, Glu and Lys
  VARIANT (23)..(23): Xaa is selected from the group consisting of Ile and Val
  VARIANT (24)..(24): Xaa is selected from the group consisting of Ala, Asn and Gln
  VARIANT (27)..(27): Xaa is selected from the group consisting of Val and Leu
  VARIANT (28)..(28): Xaa is selected from the group consisting of Arg and Ala
  VARIANT (29)..(29): Xaa is selected from the group consisting of Gly and Gln
  VARIANT (30)..(30): Xaa is selected from the group consisting of Gly and Lys
XXEGTFTSDXSXXXXXXXXXEFXXWLXXXXPSSGAPPPS

SEQ ID NO: 20 - protein, 39 aa, Artificial Sequence
  VARIANT (2)..(2): Xaa is Aib
  VARIANT (14)..(14): Xaa is Lys or Leu
  VARIANT (15)..(15): Xaa is Asp or Glu
  VARIANT (16)..(16): Xaa is Lys or Arg
  VARIANT (23)..(23): Xaa is Val or Ile
  VARIANT (27)..(27): Xaa is Ile or Leu
YXEGTFTSDYSIYXXXIAAQEFXNWLXAGGPSSGAPPPS